European Patent Application EP 4 696 320 A2, published February 18, 2026. Title: An antigen-binding molecule, a pharmaceutical composition, and a method. Applicant: CHUGAI SEIYAKU KABUSHIKI KAISHA. The sequence listing filed with the application follows.

SEQUENCE LISTING (26 sequences)

SEQ ID NO: 1 - protein, 701 aa, Macaca fascicularis
MWCIILFSLLAWVYAEPTMYGEILSPNYPQAYPSEVEKSWDIEVPEGYGIHLYFTHLDIELSENCAYDSVQIMSGDIEEGRLCGQRTSNNPYSPIVEEFQVPYNKLQVIFKSDFSNEERFTGFAAYYVATDINECTDFVDAPCSHFCNNFIGGYFCSCPPEYFLHDDMKNCGVNCSGDVFTALIGEIASPNYPKPYPENSRCEYQIRLEKGFQVVVTVRREDFDVEPADSEGNCLDSLVFVAGDQQFGPYCGRGFPGPLNIETKSNVLDIIFQTDLTGQNKGWKLRYHGDPMPCPKEETPTSVWEPAKAKYVFRDVVRITCLDGFEVVEGRVGATSFHSTCQSNGKWSNSKLKCQPVDCGIPESIENGKVEDPESTLFGSVTRYTCEEPYYYMENGGNGQYHCASNGSWVNEALSPELPKCVPVCGVPREPFEGKQRIIGGSDADIKNFPWQVFFDNPWAGGALIDEYWVLTAAHVVEGNQEPTMYVGSTSVQTSRLAKSKMLTSERVFIHPGWKLLEVPEARTNFDNDIALVQLKDPVKMGPTVAPICLPGTSSDYNLMDGDLGLIAGWGRTEKRDRALRLKAARLPVAPLRKCREVKVENPKADAGAYVFTPNMICAGGEKGMDSCKGDSGGAFAVQDPNDKTKFYVAGLVSWGPQCGTYGLYTRVQNYVDWIKKTMQENSTPSKDGGGGSDYKDDDDK

SEQ ID NO: 2 - protein, 718 aa, Macaca fascicularis
MWLLYLLVPALFCRAGGSIPIPQKLFGEVTSPLFPKPYPNSFETTTVITVPTGYRVKLVFQHFDLEPSEGCFYDYVKISADKKNLGRFCGQLGSPLGNPPGKKEFLSQGNKMLLTFHTDFSNEENGTIMFYKGFLAYYQAVDLDECASQSESGEKDPQPQCQHLCHNYVGGYFCSCRPGYELQEDRHSCQAECSSELYTEASGYISSLEYPRSYPPDLRCNYSIRVERGLTLHLKFLEPFEIDDHQQVHCPYDQLQIYANGKNIGEFCGKQRPPDFDTSSNAVDLLFFTDESGDSRGWKLRYTTEIIKCPQPKTLDEFTVIQNLQPQYQFRDYFIATCKLGYQLIEGNQVLHSFTAVCQDDGTWHRAMPRCKIKDCGQPRNLPNGAFRYTTTMGVNTYKARIQYYCHEPYYKMQTRAGSKESEQGLYTCTAQGIWKNEQKGEKIPRCLPVCGKPVNPVEQRQQIIGGQKAKMGNFPWQVFTNIHGRGGGALLGDRWILTAAHTLYPKEHEAQSNASLDVFLGHTNVEELMKLANHPIRRVSIHPDYRQDESHNFEGDIALLELENSVTLGPNLLPICLPDNETFYDLGLMGYVSGFGVMEEKIAHDLRFVRLPVANRKDCETWLRGKNRLDVFSQNMFCAGHPSLKQDACQGDAGGVFAVRDPNTDRWIATGIVSWGIGCSKGYGFYTKVLNYVDWIKKEMEEEDGGGGSHHHHHHHH

SEQ ID NO: 3 - protein, 688 aa, Homo sapiens
MWCIVLFSLLAWVYAEPTMYGEILSPNYPQAYPSEVEKSWDIEVPEGYGIHLYFTHLDIELSENCAYDSVQIISGDTEEGRLCGQRSSNNPHSPIVEEFQVPYNKLQVIFKSDFSNEERFTGFAAYYVATDINECTDFVDVPCSHFCNNFIGGYFCSCPPEYFLHDDMKNCGVNCSGDVFTALIGEIASPNYPKPYPENSRCEYQIRLEKGFQVVVTLRREDFDVEAADSAGNCLDSLVFVAGDRQFGPYCGHGFPGPLNIETKSNALDIIFQTDLTGQKKGWKLRYHGDPMPCPKEDTPNSVWEPAKAKYVFRDVVQITCLDGFEVVEGRVGATSFYSTCQSNGKWSNSKLKCQPVDCGIPESIENGKVEDPESTLFGSVIRYTCEEPYYYMENGGGGEYHCAGNGSWVNEVLGPELPKCVPVCGVPREPFEEKQRIIGGSDADIKNFPWQVFFDNPWAGGALINEYWVLTAAHVVEGNREPTMYVGSTSVQTSRLAKSKMLTPEHVFIHPGWKLLEVPEGRTNFDNDIALVRLKDPVKMGPTVSPICLPGTSSDYNLMDGDLGLISGWGRTEKRDRAVRLKAARLPVAPLRKCKEVKVEKPTADAEAYVFTPNMICAGGEKGMDSCKGDSGGAFAVQDPNDKTKFYAAGLVSWGPQCGTYGLYTRVKNYVDWIMKTMQENSTPRED

SEQ ID NO: 4 - protein, 705 aa, Homo sapiens
MWLLYLLVPALFCRAGGSIPIPQKLFGEVTSPLFPKPYPNNFETTTVITVPTGYRVKLVFQQFDLEPSEGCFYDYVKISADKKSLGRFCGQLGSPLGNPPGKKEFMSQGNKMLLTFHTDFSNEENGTIMFYKGFLAYYQAVDLDECASRSKLGEEDPQPQCQHLCHNYVGGYFCSCRPGYELQEDRHSCQAECSSELYTEASGYISSLEYPRSYPPDLRCNYSIRVERGLTLHLKFLEPFDIDDHQQVHCPYDQLQIYANGKNIGEFCGKQRPPDLDTSSNAVDLLFFTDESGDSRGWKLRYTTEIIKCPQPKTLDEFTIIQNLQPQYQFRDYFIATCKQGYQLIEGNQVLHSFTAVCQDDGTWHRAMPRCKIKDCGQPRNLPNGDFRYTTTMGVNTYKARIQYYCHEPYYKMQTRAGSRESEQGVYTCTAQGIWKNEQKGEKIPRCLPVCGKPVNPVEQRQQIIGGQKAKMGNFPWQVFTNIHGRGGGALLGDRWILTAAHTLYPKEHEAQSNASLDVFLGHTNVEELMKLGNHPIRRVSVHPDYRQDESYNFEGDIALLELENSVTLGPNLLPICLPDNDTFYDLGLMGYVSGFGVMEEKIAHDLRFVRLPVANPQACENWLRGKNRMDVFSQNMFCAGHPSLKQDACQGDAGGVFAVRDPNTDRWVATGIVSWGIGCSRGYGFYTKVLNYVDWIKKEMEEED

SEQ ID NO: 5 - protein, 279 aa, Macaca fascicularis
QVDTTKAVITLQPPWVSVFQEETVTLQCEVPRLPGSSSTQWFLNGTATQTSTPSYRITSASVKDSGEYRCQRGPSGRSDPIQLEIHRDWLLLQVSSRVFTEGEPLALRCHAWKDKLVYNVLYYQNGKAFKFFYRNSQLTILKTNISHNGAYHCSGMGKHRYTSAGVSVTVKELFPAPVLNASVTSPLLEGNLVTLSCETKLLLQRPGLQLYFSFYMGSKTLRGRNTSSEYQILTARREDSGFYWCEATTEDGNVLKRSPELELQVLGLQLPTPHHHHHH

SEQ ID NO: 6 - protein, 190 aa, Macaca fascicularis
QTAPPKAVLKLEPPWINVLREDSVTLTCGGAHSPDSDSTQWFHNGNLIPTHTQPSYRFKANNNDSGEYRCQTGRTSLSDPVHLTVLSEWLALQTPHLEFREGETIMLRCHSWKDKPLIKVTFFQNGIAKKFSHMDPNFSIPRANHSHSGDYHCTGNIGYTPYSSKPVTITVQVPSVGSSSPMGIHHHHHH

SEQ ID NO: 7 - protein, 190 aa, Macaca fascicularis
QTAPPKAVLKLEPPWINVLREDSVTLTCGGAHSPDSDSTQWFHNGNLIPTHTQPSYRFKANNNDSGEYRCQTGRTSLSDPVHLTVLSEWLALQTTHLEFREGETIMLRCHSWKDKPLIKVAFFQNGKSKNFSHMNPNFSIPQANHSHSGDYHCTGNIGYTPYSSKPVTITVQVPSVGSSSPMGIHHHHHH

SEQ ID NO: 8 - protein, 190 aa, Macaca fascicularis
QTAPPKAVLKLEPPWINVLREDSVTLTCGGAHSPDSDSTQWFHNGNLIPTHTQPSYRFKANNNDSGEYRCQTGRTSLSDPVHLTVLSEWLALQTTHLEFREGETIMLRCHSWKDKPLIKVAFFQNGISKKFSPMNPNFSIPRANHSHSGDYHCTGNIGYTPYSSKPVTITVQVPSVGSSSPMGIHHHHHH

SEQ ID NO: 9 - protein, 181 aa, Macaca fascicularis
TPAAPPKAVLKLEPPWINVLREDSVTLTCGGAHSPDSDSTQWFHNGNLIPTHTQPSYRFKANNNDSGEYRCQTGRTSLSDPVHLTVLSEWLALQTPHLEFREGETIMLRCHSWKDKPLIKVTFFQNGISKKFSHMNPNFSIPQANHSHSGDYHCTGNIGYTPYSSKPVTITVQVPHHHHHH

SEQ ID NO: 10 - protein, 194 aa, Macaca fascicularis
EDLPKAVVFLEPQWYRVLEKDRVTLKCQGAYSPEDNSTRWFHNESLISSQTSSYFIAAARVNNSGEYRCQTSLSTLSDPVQLEVHIGWLLLQAPRWVFKEEESIHLRCHSWKNTLLHKVTYLQNGKGRKYFHQNSDFYIPKATLKDSGSYFCRGLIGSKNVSSETVNITITQDLAVSSISSFFPPGYQHHHHHH

SEQ ID NO: 11 - protein, 194 aa, Macaca fascicularis
EDLPKAVVFLEPQWYRVLEKDSVTLKCQGAYSPEDNSTRWFHNESLISSQTSSYFIAAARVNNSGEYRCQTSLSTLSDPVQLEVHIGWLLLQAPRWVFKEEESIHLRCHSWKNTLLHKVTYLQNGKGRKYFHQNSDFYIPKATLKDSGSYFCRGLIGSKNVSSETVNITITQDLAVSSISSFFPPGYQHHHHHH

SEQ ID NO: 12 - protein, 115 aa, synthetic construct
  REGION 1..115: note = COS0098bb_VH
QSVEESGGRLVTPGTPLTLTCTVSGFSLTKYTVSWVRQAPGKGLEWIGIINTGGSAYYATWAKGRFTFSKTSTTVDLQITSPTTEDTATYFCARGNGDTDYTNLWGPGTLVTVSS

SEQ ID NO: 13 - protein, 106 aa, synthetic construct
  REGION 1..106: note = COS0098bb_VL
QVLTQTPSSVSEPVGGTVTINCQASENIYSALAWYQQKPGQPPKLLIYGASNLESGVPSRFKGSGSGTQFTLTISDLECADAATYYCQQYYFTSSTFGGGTKVEIK

SEQ ID NO: 14 - protein, 328 aa, synthetic construct
  REGION 1..328: note = SG1
ASTKGPSVFPLAPSSKSTSGGTAALGCLVKDYFPEPVTVSWNSGALTSGVHTFPAVLQSSGLYSLSSVVTVPSSSLGTQTYICNVNHKPSNTKVDKKVEPKSCDKTHTCPPCPAPELLGGPSVFLFPPKPKDTLMISRTPEVTCVVVDVSHEDPEVKFNWYVDGVEVHNAKTKPREEQYNSTYRVVSVLTVLHQDWLNGKEYKCKVSNKALPAPIEKTISKAKGQPREPQVYTLPPSREEMTKNQVSLTCLVKGFYPSDIAVEWESNGQPENNYKTTPPVLDSDGSFFLYSKLTVDKSRWQQGNVFSCSVMHEALHNHYTQKSLSLSP

SEQ ID NO: 15 - protein, 328 aa, synthetic construct
  REGION 1..328: note = SG1077
ASTKGPSVFPLAPSSKSTSGGTAALGCLVKDYFPEPVTVSWNSGALTSGVHTFPAVLQSSGLYSLSSVVTVPSSSLGTQTYICNVNHKPSNTKVDKRVEPKSCDKTHTCPPCPAPELWNGPSVFLFPPKPKDTLMISRTPEVTCVVVDVSDEDPEVKFNWYVDGVEVHNAKTKPREELYNSTYRVVSVLTVLHRDWLNGKEYKCKVSNTALPKPIEKTISKAKGQRREPQVYTLPPSREEMTKNQVSLTCLVKGFYPSDIAVEWESNGQPENNYKTTPPVLDSDGSFFLYSKLTVDKSRWQQGNVFSCSVLHEALHAHTTRKELSLSP

SEQ ID NO: 16 - protein, 328 aa, synthetic construct
  REGION 1..328: note = SG1148
ASTKGPSVFPLAPSSKSTSGGTAALGCLVKDYFPEPVTVSWNSGALTSGVHTFPAVLQSSGLYSLSSVVTVPSSSLGTQTYICNVNHKPSNTKVDKKVEPKSCDKTHTCPPCPAPELLGGPSVFLFPPKPKDTLMISRTPEVTCVVVDVSHEDPEVKFNWYVDGVEVHNAKTKPREEQYNSTYRVVSVLTVLHQDWLNGKEYKCEVSNKALPAPIEKTISKAKGQPREPQVYTLPPSREEMTKNQVSLTCLVKGFYPSDIAVEWESNGQPENNYKTTPPVLDSDGSFFLYSKLTVDKSRWQQGNVFSCSVMHEALHNHYTQKSLSLSP

SEQ ID NO: 17 - protein, 107 aa, synthetic construct
  REGION 1..107: note = K0MC
RTVAAPSVFIFPPSDEQLKSGTASVVCLLNNFYPREAKVQWKVDNALQSGNSQESVTEQDSKDCTYSLSSTLTLSKADYEKHKVYACEVTHQGLSSPVTKSFNRGEC

SEQ ID NO: 18 - protein, 118 aa, synthetic construct
  REGION 1..118: note = COS0098pHv1_VH
QVQLVQSGAEVKKPGSSVKVSCKASGHTFSKYTVSWIRQPPGKGLEWIGIINTGGSAYPATWAKGRVTITADESTSTAYMELSSLRSEDTAVYYCARGAGDTDYTNLWGQGTLVTVSS

SEQ ID NO: 19 - protein, 107 aa, synthetic construct
  REGION 1..107: note = COS0098pHv1_VL
DIQMTQSPSSLSASVGDRVTITCQASENIYSALAWYQQKPGQPPKLLIYGASQLESGVPSRFSGSGSGTDFTLTISSLQPEDFATYYCQQYYFTSHTFGQGTKVEIK

SEQ ID NO: 20 - protein, 5 aa, synthetic construct
  REGION 1..5: note = COS0098pHv1_HCDR1
KYTVS

SEQ ID NO: 21 - protein, 16 aa, synthetic construct
  REGION 1..16: note = COS0098pHv1_HCDR2
IINTGGSAYPATWAKG

SEQ ID NO: 22 - protein, 10 aa, synthetic construct
  REGION 1..10: note = COS0098pHv1_HCDR3
GAGDTDYTNL

SEQ ID NO: 23 - protein, 11 aa, synthetic construct
  REGION 1..11: note = COS0098pHv1_LCDR1
QASENIYSALA

SEQ ID NO: 24 - protein, 7 aa, synthetic construct
  REGION 1..7: note = COS0098pHv1_LCDR2
GASQLES

SEQ ID NO: 25 - protein, 9 aa, synthetic construct
  REGION 1..9: note = COS0098pHv1_LCDR3
QQYYFTSHT

SEQ ID NO: 26 - protein, 107 aa, synthetic construct [sequence omitted]